European Patent Application EP 4 302 771 A1, published January 10, 2024. Title: lymphangiogenesis promoting factor expressing fibroblast and pahrmaceutical composition comprising the same. Applicant: Metcela Inc. The sequence listing filed with the application follows.

SEQUENCE LISTING (28 sequences)

SEQ ID NO: 1 - DNA, 1492 bp, Homo sapiens
actcagtggtttcttggtgacactggatagaacagctcaagccttgccacttcgggcttctcactgcagctgggcttggacttcggagttttgccattgccagtgggacgtctgagactttctccttcaagtacttggcagatcactctcttagcagggtctgcgcttcgcagccgggatgaagctggtttccgtcgccctgatgtacctgggttcgctcgccttcctaggcgctgacaccgctcggttggatgtcgcgtcggagtttcgaaagaagtggaataagtgggctctgagtcgtgggaagagggaactgcggatgtccagcagctaccccaccgggctcgctgacgtgaaggccgggcctgcccagacccttattcggccccaggacatgaagggtgcctctcgaagccccgaagacagcagtccggatgccgcccgcatccgagtcaagcgctaccgccagagcatgaacaacttccagggcctccggagctttggctgccgcttcgggacgtgcacggtgcagaagctggcacaccagatctaccagttcacagataaggacaaggacaacgtcgcccccaggagcaagatcagcccccagggctacggccgccggcgccggcgctccctgcccgaggccggcccgggtcggactctggtgtcttctaagccacaagcacacggggctccagcccccccgagtggaagtgctccccactttctttaggatttaggcgcccatggtacaaggaatagtcgcgcaagcatcccgctggtgcctcccgggacgaaggacttcccgagcggtgtggggaccgggctctgacagccctgcggagaccctgagtccgggaggcaccgtccggcggcgagctctggctttgcaagggcccctccttctgggggcttcgcttccttagccttgctcaggtgcaagtgccccagggggcggggtgcagaagaatccgagtgtttgccaggcttaaggagaggagaaactgagaaatgaatgctgagacccccggagcaggggtctgagccacagccgtgctcgcccacaaactgatttctcacggcgtgtcaccccaccagggcgcaagcctcactattacttgaactttccaaaacctaaagaggaaaagtgcaatgcgtgttgtacatacagaggtaactatcaatatttaagtttgttgctgtcaagattttttttgtaacttcaaatatagagatatttttgtacgttatatattgtattaagggcattttaaaagcaattatattgtcctcccctattttaagacgtgaatgtctcagcgaggtgtaaagttgttcgccgcgtggaatgtgagtgtgtttgtgtgcatgaaagagaaagactgattacctcctgtgtggaagaaggaaacaccgagtctctgtataatctatttacataaaatgggtgatatgcgaacagcaaaccaataaactgtctcaatgctga

SEQ ID NO: 2 - DNA, 1724 bp, Homo sapiens
agctctgcgaggggccggagcgcggcggagccatgcagtacccgcaccccgggccggcggcgggcgccgtgggggtgccgctgtacgcgcccacgccgctgctgcaacccgcacacccgacgcccttttacatcgaggacatcctgggccgcgggcccgccgcgcccacgcccgcccccacgctgccgtcccccaactcctccttcaccagcctcgtgtccccctaccggaccccggtgtacgagcccacgccgatccatccagccttctcgcaccactccgccgccgcgctggccgctgcctacggacccggcggcttcgggggccctctgtaccccttcccgcggacggtgaacgactacacgcacgccctgctccgccacgaccccctgggcaaacctctactctggagccccttcttgcagaggcctctgcataaaaggaaaggcggccaggtgagattctccaacgaccagaccatcgagctggagaagaaattcgagacgcagaaatatctctctccgcccgagaggaagcgtctggccaagatgctgcagctcagcgagagacaggtcaaaacctggtttcagaatcgacgcgctaaatggaggagactaaaacaggagaaccctcaaagcaataaaaaagaagaactggaaagtttggacagttcctgtgatcagaggcaagatttgcccagtgaacagaataaaggtgcttctttggatagctctcaatgttcgccctcccctgcctcccaggaagaccttgaatcagagatttcagaggattctgatcaggaagtggacattgagggcgataaaagctattttaatgctggatgatgaccactggcattggcatgttcagaaaactggatttaggaataatgttttgctacagaaaatcttcatagaagaactggaaggctatataagaaagggaatcaattctctggtattctggaaacctaaaaatatttggtgcactgctcaattaacaaacctacatggagaccttaattttgacttaacaaatagtttatgtactgctcttaggttgttttgataaagtgacattatagtgattaaattcttccccctttaaaaaaacagttagtggttttcactatttataaaaaattaattttgaactttttgttaaatttttaagttatagctttaaaggttttaataggaccttcttgaacgacttttctgtaatctgtttatctcccacttaatggaaaggcaaaggggtaccccaaatccagaggtgcctacatttcaggcagccttggagtattttaaaaggaaaacattctttacttttatatgacattcttatactgctgtctcaaatccaaaaacatttcagagctcttgtctcagagatgtgtgttctttttgtcagagatatggttgatgagaatcttaaatgcttgttttgcactatcacttagtacctgtttgaccaaggtgttaaggggatagtacctcccaattcaagcagagaaactgacctgactaaagttaatcgcagatgaactagaagtcacaggttaattaaatgtaagtagattgtagatactgttttatatcaaacaatgtttataatgtgtatatagaattgttcactgtaaaaaaaatggccaaaatgtgttttttttttaataagtaacttgactataaaataaagccgtccgtgggacgactgacctcgtt

SEQ ID NO: 3 - DNA, 1812 bp, Homo sapiens
accgccgagaccgcgtccgccccgcgagcacagagcctcgcctttgccgatccgccgcccgtccacacccgccgccagctcaccatggatgatgatatcgccgcgctcgtcgtcgacaacggctccggcatgtgcaaggccggcttcgcgggcgacgatgccccccgggccgtcttcccctccatcgtggggcgccccaggcaccagggcgtgatggtgggcatgggtcagaaggattcctatgtgggcgacgaggcccagagcaagagaggcatcctcaccctgaagtaccccatcgagcacggcatcgtcaccaactgggacgacatggagaaaatctggcaccacaccttctacaatgagctgcgtgtggctcccgaggagcaccccgtgctgctgaccgaggcccccctgaaccccaaggccaaccgcgagaagatgacccagatcatgtttgagaccttcaacaccccagccatgtacgttgctatccaggctgtgctatccctgtacgcctctggccgtaccactggcatcgtgatggactccggtgacggggtcacccacactgtgcccatctacgaggggtatgccctcccccatgccatcctgcgtctggacctggctggccgggacctgactgactacctcatgaagatcctcaccgagcgcggctacagcttcaccaccacggccgagcgggaaatcgtgcgtgacattaaggagaagctgtgctacgtcgccctggacttcgagcaagagatggccacggctgcttccagctcctccctggagaagagctacgagctgcctgacggccaggtcatcaccattggcaatgagcggttccgctgccctgaggcactcttccagccttccttcctgggcatggagtcctgtggcatccacgaaactaccttcaactccatcatgaagtgtgacgtggacatccgcaaagacctgtacgccaacacagtgctgtctggcggcaccaccatgtaccctggcattgccgacaggatgcagaaggagatcactgccctggcacccagcacaatgaagatcaagatcattgctcctcctgagcgcaagtactccgtgtggatcggcggctccatcctggcctcgctgtccaccttccagcagatgtggatcagcaagcaggagtatgacgagtccggcccctccatcgtccaccgcaaatgcttctaggcggactatgacttagttgcgttacaccctttcttgacaaaacctaacttgcgcagaaaacaagatgagattggcatggctttatttgttttttttgttttgttttggttttttttttttttttggcttgactcaggatttaaaaactggaacggtgaaggtgacagcagtcggttggagcgagcatcccccaaagttcacaatgtggccgaggactttgattgcacattgttgtttttttaatagtcattccaaatatgagatgcgttgttacaggaagtcccttgccatcctaaaagccaccccacttctctctaaggagaatggcccagtcctctcccaagtccacacaggggaggtgatagcattgctttcgtgtaaattatgtaatgcaaaatttttttaatcttcgccttaatacttttttattttgttttattttgaatgatgagccttcgtgcccccccttcccccttttttgtcccccaacttgagatgtatgaaggcttttggtctccctgggagtgggtggaggcagccagggcttacctgtacactgacttgagaccagttgaataaaagtgcacaccttaaaaatga

SEQ ID NO: 4 - DNA, 20 bp, Artificial Sequence
  human ADM Forward Primer
atgtacctgggttcgctcgc

SEQ ID NO: 5 - DNA, 20 bp, Artificial Sequence
  human ADM Reverse Primer
ccacgactcagagcccactt

SEQ ID NO: 6 - DNA, 20 bp, Artificial Sequence
  human HHEX Forward Primer
agcgagagacaggtcaaaac

SEQ ID NO: 7 - DNA, 21 bp, Artificial Sequence
  human HHEX Reverse Primer
ctgttcactgggcaaatcttg

SEQ ID NO: 8 - DNA, 20 bp, Artificial Sequence
  human ACTB Forward Primer
accttctacaatgagctgcg

SEQ ID NO: 9 - DNA, 21 bp, Artificial Sequence
  human ACTB Reverse Primer
cctggatagcaacgtacatgg

SEQ ID NO: 10 - DNA, 23 bp, Artificial Sequence
  human ADM Probe
ttcgaaactccgacgcgacatcc

SEQ ID NO: 11 - DNA, 25 bp, Artificial Sequence
  human HHEX Probe
cctccatttagcgcgtcgattctga

SEQ ID NO: 12 - DNA, 24 bp, Artificial Sequence
  human ACTB Probe
atctgggtcatcttctcgcggttg

SEQ ID NO: 13 - DNA, 2259 bp, Homo sapiens
atgccctgcccctgcgcccgccgccgccgccgccgccgctcagcccggcgcgctctggaggatcctgcgccgcggcgctcccgggccccgccgccgccagccgccccgccgccctcctcccgcccccggcaccgccgccagcgcccccgccgcagcgcccgcggcccggctcctctcacttcggggaaggggagggaggagggggacgagggctctggcgggtttggaggggctgaacatcgcggggtgttctggtgtcccccgccccgcctctccaaaaagctacaccgacgcggaccgcggcggcgtcctccctcgccctcgcttcacctcgcgggctccgaatgcggggagctcggatgtccggtttcctgtgaggcttttacctgacacccgccgcctttccccggcactggctgggagggcgccctgcaaagttgggaacgcggagccccggacccgctcccgccgcctccggctcgcccagggggggtcgccgggaggagcccgggggagagggaccaggaggggcccgcggcctcgcaggggcgcccgcgcccccacccctgcccccgccagcggaccggtcccccacccccggtccttccaccatgcacttgctgggcttcttctctgtggcgtgttctctgctcgccgctgcgctgctcccgggtcctcgcgaggcgcccgccgccgccgccgccttcgagtccggactcgacctctcggacgcggagcccgacgcgggcgaggccacggcttatgcaagcaaagatctggaggagcagttacggtctgtgtccagtgtagatgaactcatgactgtactctacccagaatattggaaaatgtacaagtgtcagctaaggaaaggaggctggcaacataacagagaacaggccaacctcaactcaaggacagaagagactataaaatttgctgcagcacattataatacagagatcttgaaaagtattgataatgagtggagaaagactcaatgcatgccacgggaggtgtgtatagatgtggggaaggagtttggagtcgcgacaaacaccttctttaaacctccatgtgtgtccgtctacagatgtgggggttgctgcaatagtgaggggctgcagtgcatgaacaccagcacgagctacctcagcaagacgttatttgaaattacagtgcctctctctcaaggccccaaaccagtaacaatcagttttgccaatcacacttcctgccgatgcatgtctaaactggatgtttacagacaagttcattccattattagacgttccctgccagcaacactaccacagtgtcaggcagcgaacaagacctgccccaccaattacatgtggaataatcacatctgcagatgcctggctcaggaagattttatgttttcctcggatgctggagatgactcaacagatggattccatgacatctgtggaccaaacaaggagctggatgaagagacctgtcagtgtgtctgcagagcggggcttcggcctgccagctgtggaccccacaaagaactagacagaaactcatgccagtgtgtctgtaaaaacaaactcttccccagccaatgtggggccaaccgagaatttgatgaaaacacatgccagtgtgtatgtaaaagaacctgccccagaaatcaacccctaaatcctggaaaatgtgcctgtgaatgtacagaaagtccacagaaatgcttgttaaaaggaaagaagttccaccaccaaacatgcagctgttacagacggccatgtacgaaccgccagaaggcttgtgagccaggattttcatatagtgaagaagtgtgtcgttgtgtcccttcatattggaaaagaccacaaatgagctaagattgtactgttttccagttcatcgattttctattatggaaaactgtgttgccacagtagaactgtctgtgaacagagagacccttgtgggtccatgctaacaaagacaaaagtctgtctttcctgaaccatgtggataactttacagaaatggactggagctcatctgcaaaaggcctcttgtaaagactggttttctgccaatgaccaaacagccaagattttcctcttgtgatttctttaaaagaatgactatataatttatttccactaaaaatattgtttctgcattcatttttatagcaacaacaattggtaaaactcactgtgatcaatatttttatatcatgcaaaatatgtttaaaataaaatgaaaattgtattataa

SEQ ID NO: 14 - DNA, 1881 bp, Mus musculus
ccgccaccgagggcagttcggatgtccggtttcctgtgaggctcgtacctgacacccgggagcctctcccccgtgagggctgccagagccgagggcaaaagttgcgagccgccgagtcccgggagacgctcgcccaggggggtccccgggaggaaaccacgggacagggaccaggagaggacctcagcctcacgccccagcctgcgccagccaacggaccggcctccctgctcccggtccatccaccatgcacttgctgtgcttcttgtctctggcgtgttccctgctcgccgctgcgctgatccccagtccgcgcgaggcgcccgccaccgtcgccgccttcgagtcgggactgggcttctcggaagcggagcccgacgggggcgaggtcaaggcttttgaaggcaaagacctggaggagcagttgcggtctgtgtccagcgtagatgagctgatgtctgtcctgtacccagactactggaaaatgtacaagtgccagctgcggaaaggcggctggcagcagcccaccctcaataccaggacaggggacagtgtaaaatttgctgctgcacattataacacagagatcctgaaaagtattgataatgagtggagaaagactcaatgcatgccacgtgaggtgtgtatagatgtggggaaggagtttggagcagccacaaacaccttctttaaacctccatgtgtgtccgtctacagatgtgggggttgctgcaacagcgaggggctgcagtgcatgaacaccagcacaggttacctcagcaagacgttgtttgaaattacagtgcctctctcacaaggccccaaaccagtcacaatcagttttgccaatcacacttcctgccggtgcatgtctaaactggatgtttacagacaagttcattcaattattagacgttctctgccagcaacattaccacagtgtcaggcagctaacaagacatgtccaacaaactatgtgtggaataactacatgtgccgatgcctggctcagcaggattttatcttttattcaaatgttgaagatgactcaaccaatggattccatgatgtctgtggacccaacaaggagctggatgaagacacctgtcagtgtgtctgcaagggggggcttcggccatctagttgtggaccccacaaagaactagatagagactcatgtcagtgtgtctgtaaaaacaaacttttccctaattcatgtggagccaacagggaatttgatgagaatacatgtcagtgtgtatgtaaaagaacgtgtccaagaaatcagcccctgaatcctgggaaatgtgcctgtgaatgtacagaaaacacacagaagtgcttccttaaagggaagaagttccaccatcaaacatgcagttgttacagaagaccgtgtgcgaatcgactgaagcattgtgatccaggactgtcctttagtgaagaagtatgccgctgtgtcccatcgtattggaaaaggccacatctgaactaagatcataccagttttcagtccaccattttactctcttgaagaactgttgccacattagcactgtctatgcacagaaagactctgtgggaccatggtaacagaggcccaagtctgtgtttattgaaccatgtggattactgcgggagaggactggcactcatgtgcaaaaaaacctcttcaaagactggttttctgccagggaccagacagctgaggtttttctcttgtgatttaaaaaaagaatgactatataatttatttccactaaaaatattgttcctgcattcatttttatagcaataacaattggtaaagctcactgtgatcagtatttttataacatgcaaaactatgtttaaaataaaatgaaaattgtattataagct

SEQ ID NO: 15 - DNA, 1394 bp, Mus musculus
agtcagtggtttcttggtgacactagacagagcaactccagcgttaccgctcccgctcctggtttctcggcttctcatcgcagtcaatcttggactttggggttttgctactgtcagaaggacttctttctgcttcaagtgcttgacaacgcacccctttatcagggtatcagagcatcgccacagaatgaagctggtttccatcaccctgatgttattgggttcactcgctttcctaggcgcggacactgcagggccagatactccttcgcagttccgaaagaagtggaataagtgggcgctaagtcgtgggaagagggaactacaagcatccagcagctaccctacgggactcgctgatgagacgacagttcctacccagactcttgatccattcctggacgagcagaacacaactggccccctacaagccagcaatcagagcgaagcccacattcgtgtcaaacgctaccgccagagcatgaaccagggttcccgcagcaatggatgccgcttcgggacctgcacatttcagaaattggcccaccagatctaccagctaacagacaaagacaaggacggcatggctcccagaaacaagatcagccctcaaggctatggccgccggcgccggcgttccctgctggaggtcctccggtcccggactgtggagtcctcccaggagcagacacacacagccccaggcccctgggcgcacatctccagactctttaggatataggtgcgggtgacagcattgaacagtcgggcgagtatcccgttggcgcctgcggaatcagagaacttcgcaccggggcggactgagacaatcctgcagagatctgcctggctgcccctaggggaggcagaggaacccaagaccaagccaggctcatgccagaaaccgagacttacaggctgatactctccgggcaggggtctgagccactgccttgcccgctcataaactggtttctcacggggcataagcctcattactacttgaactttccaaaacctagcgaggaacgtgcaatgcttgttgtccagccaaaggtaactatagtatttaagtttgttgctgtcaaggtttttttttttgtaacttcaaatatatagagatatttttgtacgttatatattgtattaagggcattttaaagtgattatattgtcaccttcccctattttaagacgtgaatgtctcagcaaggtgtaaggttgtttggttccgtgtgtgtgtgtgtgtgtgtgtgtgtgtgtgtgtgtgtgtaaggtggagagcgcctgattatcgcctgtggatgaagaaaaaacattgtgtttcctataatctatttacataaaatatgtgatctgggaaaaagcaaaccaataaactgtctcaatgctga

SEQ ID NO: 16 - DNA, 1296 bp, Mus musculus
aacccttaagagggatgctgcccttaccccggggtcccagcttaggttcatcaggtaaactcaggagagtgtttcctcgtcccgtagacaaaatggtgaaggtcggtgtgaacggatttggccgtattgggcgcctggtcaccagggctgccatttgcagtggcaaagtggagattgttgccatcaacgaccccttcattgacctcaactacatggtctacatgttccagtatgactccactcacggcaaattcaacggcacagtcaaggccgagaatgggaagcttgtcatcaacgggaagcccatcaccatcttccaggagcgagaccccactaacatcaaatggggtgaggccggtgctgagtatgtcgtggagtctactggtgtcttcaccaccatggagaaggccggggcccacttgaagggtggagccaaaagggtcatcatctccgccccttctgccgatgcccccatgtttgtgatgggtgtgaaccacgagaaatatgacaactcactcaagattgtcagcaatgcatcctgcaccaccaactgcttagcccccctggccaaggtcatccatgacaactttggcattgtggaagggctcatgaccacagtccatgccatcactgccacccagaagactgtggatggcccctctggaaagctgtggcgtgatggccgtggggctgcccagaacatcatccctgcatccactggtgctgccaaggctgtgggcaaggtcatcccagagctgaacgggaagctcactggcatggccttccgtgttcctacccccaatgtgtccgtcgtggatctgacgtgccgcctggagaaacctgccaagtatgatgacatcaagaaggtggtgaagcaggcatctgagggcccactgaagggcatcttgggctacactgaggaccaggttgtctcctgcgacttcaacagcaactcccactcttccaccttcgatgccggggctggcattgctctcaatgacaactttgtcaagctcatttcctggtatgacaatgaatacggctacagcaacagggtggtggacctcatggcctacatggcctccaaggagtaagaaaccctggaccacccaccccagcaaggacactgagcaagagaggccctatcccaactcggcccccaacactgagcatctccctcacaatttccatcccagacccccataataacaggaggggcctagggagccctccctactctcttgaataccatcaataaagttcgctgcacccacaaaaaaaaaaaaaaaaaaaaaa

SEQ ID NO: 17 - DNA, 24 bp, Artificial Sequence
  human VEGF-C Forward Primer
gctacctcagcaagacgttatttg

SEQ ID NO: 18 - DNA, 20 bp, Artificial Sequence
  human VEGF-C Reverse Primer
atcggcaggaagtgtgattg

SEQ ID NO: 19 - DNA, 19 bp, Artificial Sequence
  mouse VEGF-C Forward Primer
gcttcttgtctctggcgtg

SEQ ID NO: 20 - DNA, 18 bp, Artificial Sequence
  mouse VEGF-C Reverse Primer
gacacagaccgcaactgc

SEQ ID NO: 21 - DNA, 20 bp, Artificial Sequence
  mouse ADM Forward Primer
gggccagatactccttcgca

SEQ ID NO: 22 - DNA, 20 bp, Artificial Sequence
  mouse ADM Reverse Primer
ctggcggtagcgtttgacac

SEQ ID NO: 23 - DNA, 19 bp, Artificial Sequence
  mouse GAPDH Forward Primer
gaggccggtgctgagtatg

SEQ ID NO: 24 - DNA, 19 bp, Artificial Sequence
  mouse GAPDH Reverse Primer
acccttttggctccaccct

SEQ ID NO: 25 - DNA, 28 bp, Artificial Sequence
  human VEGF-C Probe
aattacagtgcctctctctcaaggcccc

SEQ ID NO: 26 - DNA, 29 bp, Artificial Sequence
  mouse VEGF-C Probe
tctttgccttcaaaagccttgacctcgcc

SEQ ID NO: 27 - DNA, 27 bp, Artificial Sequence
  mouse ADM Probe
tccgaaagaagtggaataagtgggcgc

SEQ ID NO: 28 - DNA, 19 bp, Artificial Sequence
  mouse GAPDH Probe
tcaagtgggccccggcctt